European Patent Application EP 4 230 721 A1, published August 23, 2023. Title: Microorganisms with reduced competence. Applicant: Evonik Operations GmbH. The sequence listing filed with the application follows.

SEQUENCE LISTING (12 sequences)

SEQ ID NO: 1 - DNA, 579 bp, Bacillus velezensis
atgtgccagaaaacacatgcacccttagaaagctacgaagtaaatcgttcaaccatcgctgttttgcctgaggaaatagacggtaaaatggggtcgaaggtcattgaaaaagactgcattctgtatgtcagcatgaagccgattcacatcatcgacagaagctgccgctactttggctccagctatgccgggagaaaagcgggaacatatgaagcgattaaaatttctcacaagccgccgattatggtggacccttcaaatcacatctttttattccctacactttcttctgcaaggcctcaatgcggctggatatctcatgtgcacgttaaagattttcaaccgacggcatttgatgacacagcggtcacgttctcaaacggcaaaacgatggaactggaagtatcctatcattcttttgaaaatcaggtttacagaaccgcatatctcagaaccacttttcaggacaggatgggcagtcatgtcccgaagcggcaggaattcatgctgtatccgaaagaagagcggacaagaatgatctacgactttattttgcgggagctgggggagagatattag

SEQ ID NO: 2 - DNA, 579 bp, Bacillus velezensis
atgtgccagtaaacacatgcacccttagaaagcttctaagtaaatcgttcaaccatcgctgttttgcctgaggaaatagacggtaaaatggggtcgaaggtcattgaaaaagactgcattctgtatgtcagcatgaagccgattcacatcatcgacagaagctgccgctactttggctccagctatgccgggagaaaagcgggaacatatgaagcgattaaaatttctcacaagccgccgattatggtggacccttcaaatcacatctttttattccctacactttcttctgcaaggcctcaatgcggctggatatctcatgtgcacgttaaagattttcaaccgacggcatttgatgacacagcggtcacgttctcaaacggcaaaacgatggaactggaagtatcctatcattcttttgaaaatcaggtttacagaaccgcatatctcagaaccacttttcaggacaggatgggcagtcatgtcccgaagcggcaggaattcatgctgtatccgaaagaagagcggacaagaatgatctacgactttattttgcgggagctgggggagagatattag

SEQ ID NO: 3 - DNA, 20 bp, Bacillus velezensis
cacaatcactggccgcaatg

SEQ ID NO: 4 - DNA, 21 bp, Bacillus velezensis
tagacttccctccttccgcac

SEQ ID NO: 5 - DNA, 24 bp, Bacillus velezensis
atcattaatacggcctctattacc

SEQ ID NO: 6 - DNA, 38 bp, Bacillus velezensis
ctttctaagggtgcatgtgtttactggcacataatgtg

SEQ ID NO: 7 - DNA, 37 bp, Bacillus velezensis
tgcacccttagaaagcttctaagtaaatcgttcaacc

SEQ ID NO: 8 - DNA, 20 bp, Bacillus velezensis
gtgcaccgaatcagtccatc

SEQ ID NO: 9 - DNA, 22 bp, Bacillus velezensis
tccggatggtatacgaagtcag

SEQ ID NO: 10 - DNA, 30 bp, Bacillus velezensis
tcaatgtgtaatagatgttatgcgatagcc

SEQ ID NO: 11 - DNA, 40 bp, Bacillus velezensis
tctattacacattgaagctgtcttttaacgcccgaatgag

SEQ ID NO: 12 - DNA, 22 bp, Bacillus velezensis
tccagcggaatgaaagacagtg